European Patent Specification EP 3 796 912 B1, published February 15, 2023. Title: ANTIPROLIFERATIVE COMPOUNDS AND BISPECIFIC ANTIBODY AGAINST BCMA AND CD3 FOR COMBINED USE. Applicant: Celgene Corporation. Application TBA. The sequence listing filed with the application follows.

SEQUENCE LISTING (57 sequences)

SEQ ID NO: 1 - protein, 5 aa, Mus musculus
TYAMN

SEQ ID NO: 2 - protein, 19 aa, Mus musculus
RIRSKYNNYATYYADSVKG

SEQ ID NO: 3 - protein, 14 aa, Mus musculus
HGNFGNSYVSWFAY

SEQ ID NO: 4 - protein, 14 aa, Mus musculus
GSSTGAVTTSNYAN

SEQ ID NO: 5 - protein, 7 aa, Mus musculus
GTNKRAP

SEQ ID NO: 6 - protein, 9 aa, Mus musculus
ALWYSNLWV

SEQ ID NO: 7 - protein, 125 aa, Mus musculus
EVQLLESGGGLVQPGGSLRLSCAASGFTFSTYAMNWVRQAPGKGLEWVSRIRSKYNNYATYYADSVKGRFTISRDDSKNTLYLQMNSLRAEDTAVYYCVRHGNFGNSYVSWFAYWGQGTLVTVSS

SEQ ID NO: 8 - protein, 109 aa, Mus musculus
QAVVTQEPSLTVSPGGTVTLTCGSSTGAVTTSNYANWVQEKPGQAFRGLIGGTNKRAPGTPARFSGSLLGGKAALTLSGAQPEDEAEYYCALWYSNLWVFGGGTKLTVL

SEQ ID NO: 9 - protein, 116 aa, Artificial Sequence
  83A10 Heavy Chain Variable region (VH)
EVQLLESGGGLVQPGGSLRLSCAASGFTFSSYAMSWVRQAPGKGLEWVSAISGSGGSTYYADSVKGRFTISRDNSKNTLYLQMNSLRAEDTAVYYCAKVLGWFDYWGQGTLVTVSS

SEQ ID NO: 10 - protein, 116 aa, Artificial Sequence
  Mab21/Mab22/Mab42 Heavy Chain Variable region
EVQLLESGGGLVQPGGSLRLSCAASGFTFSDNAMGWVRQAPGKGLEWVSAISGPGSSTYYADSVKGRFTISRDNSKNTLYLQMNSLRAEDTAVYYCAKVLGWFDYWGQGTLVTVSS

SEQ ID NO: 11 - protein, 109 aa, Artificial Sequence
  83A10 Light Chain Variable region (VL)
EIVLTQSPGTLSLSPGERATLSCRASQSVSSSYLAWYQQKPGQAPRLLIYGASSRATGIPDRFSGSGSGTDFTLTISRLEPEDFAVYYCQQYGYPPDFTFGQGTKVEIK

SEQ ID NO: 12 - protein, 109 aa, Artificial Sequence
  Mab21/Mab27/Mab33/Mab39 Light Chain Variable region
EIVLTQSPGTLSLSPGERATLSCRASQSVSEYYLAWYQQKPGQAPRLLIEHASTRATGIPDRFSGSGSGTDFTLTISRLEPEDFAVYYCQQYGYPPDFTFGQGTKVEIK

SEQ ID NO: 13 - protein, 109 aa, Artificial Sequence
  Mab22 Light Chain Variable region (VL)
EIVLTQSPGTLSLSPGERATLSCRASQSVSSYYLAWYQQKPGQAPRLLISGAGSRATGIPDRFSGSGSGTDFTLTISRLEPEDFAVYYCQQYGYPPDFTFGQGTKVEIK

SEQ ID NO: 14 - protein, 109 aa, Artificial Sequence
  Mab42 Light Chain Variable region (VL)
EIVLTQSPGTLSLSPGERATLSCRASQSVSDEYLSWYQQKPGQAPRLLIHSASTRATGIPDRFSGSGSGTDFTLAISRLEPEDFAVYYCQQYGYPPDFTFGQGTKVEIK

SEQ ID NO: 15 - protein, 5 aa, Homo sapiens
  83A10 CDR1H
SYAMS

SEQ ID NO: 16 - protein, 17 aa, Homo sapiens
  83A10 CDR2H
AISGSGGSTYYADSVKG

SEQ ID NO: 17 - protein, 7 aa, Homo sapiens
  83A10/Mab21/Mab22/Mab42/Mab27/Mab33/Mab39 CDR3H
VLGWFDY

SEQ ID NO: 18 - protein, 13 aa, Homo sapiens
  83A10 CDR1L
RASQSVSSSYLAW

SEQ ID NO: 19 - protein, 8 aa, Homo sapiens
  83A10 CDR2L
YGASSRAT

SEQ ID NO: 20 - protein, 10 aa, Homo sapiens
  83A10/Mab21/Mab22/Mab42 CDR3L
QQYGYPPDFT

SEQ ID NO: 21 - protein, 5 aa, Artificial Sequence
  Mab21/Mab22/Mab42 CDR1H
DNAMG

SEQ ID NO: 22 - protein, 17 aa, Artificial Sequence
  Mab21/Mab22/Mab42 CDR2H
AISGPGSSTYYADSVKG

SEQ ID NO: 23 - protein, 13 aa, Artificial Sequence
  Mab21 CDR1L
RASQSVSEYYLAW

SEQ ID NO: 24 - protein, 8 aa, Artificial Sequence
  Mab21 CDR2L
EHASTRAT

SEQ ID NO: 25 - protein, 13 aa, Artificial Sequence
  Mab22 CDR1L
RASQSVSSYYLAW

SEQ ID NO: 26 - protein, 8 aa, Artificial Sequence
  Mab22 CDR2L
SGAGSRAT

SEQ ID NO: 27 - protein, 13 aa, Artificial Sequence
  Mab42 CDR1L
RASQSVSDEYLSW

SEQ ID NO: 28 - protein, 8 aa, Artificial Sequence
  Mab42 CDR2L
HSASTRAT

SEQ ID NO: 29 - protein, 5 aa, Artificial Sequence
  Mab27 CDR1H
SAPMG

SEQ ID NO: 30 - protein, 16 aa, Artificial Sequence
  Mab27 CDR2H
AISYIGHTYYADSVKG

SEQ ID NO: 31 - protein, 12 aa, Artificial Sequence
  Mab27/Mab33/Mab39 CDR1L
RASQSVSEYYLA

SEQ ID NO: 32 - protein, 7 aa, Artificial Sequence
  Mab27/Mab33/Mab39 CDR2L
HASTRAT

SEQ ID NO: 33 - protein, 10 aa, Artificial Sequence
  Mab27/Mab33/Mab39 CDR3L
QQYGYPPDFT

SEQ ID NO: 34 - protein, 5 aa, Artificial Sequence
  Mab33 CDR1H
TNAMG

SEQ ID NO: 35 - protein, 17 aa, Artificial Sequence
  Mab33 CDR2H
AINRFGGSTYYADSVKG

SEQ ID NO: 36 - protein, 5 aa, Artificial Sequence
  Mab39 CDR1H
QNAMG

SEQ ID NO: 37 - protein, 17 aa, Artificial Sequence
  Mab39 CDR2H
AISPTGFSTYYADSVKG

SEQ ID NO: 38 - protein, 115 aa, Artificial Sequence
  Mab27 VH
EVQLLESGGGLVQPGGSLRLSCAASGFTFSSAPMGWVRQAPGKGLEWVSAISYIGHTYYADSVKGRFTISRDNSKNTLYLQMNSLRAEDTAVYYCAKVLGWFDYWGQGTLVTVSS

SEQ ID NO: 39 - protein, 116 aa, Artificial Sequence
  Mab33 VH
EVQLLESGGGLVQPGGSLRLSCAASGFTFYTNAMGWVRQAPGKGLEWVSAINRFGGSTYYADSVKGRFTISRDNSKNTLYLQMNSLRAEDTAVYYCAKVLGWFDYWGQGTLVTVSS

SEQ ID NO: 40 - protein, 116 aa, Artificial Sequence
  Mab39 VH
EVQLLESGGGLVQPGGSLRLSCAASGFTFTQNAMGWVRQAPGKGLEWVSAISPTGFSTYYADSVKGRFTISRDNSKNTLYLQMNSLRAEDTAVYYCAKVLGWFDYWGQGTLVTVSS

SEQ ID NO: 41 - protein, 103 aa, Artificial Sequence
  83A10/Mab21/Mab22/Mab42 BCMA CH1
ASTKGPSVFPLAPSSKSTSGGTAALGCLVEDYFPEPVTVSWNSGALTSGVHTFPAVLQSSGLYSLSSVVTVPSSSLGTQTYICNVNHKPSNTKVDEKVEPKSC

SEQ ID NO: 42 - protein, 107 aa, Artificial Sequence
  83A10/Mab21/Mab22/Mab42 BCMA CL
RTVAAPSVFIFPPSDRKLKSGTASVVCLLNNFYPREAKVQWKVDNALQSGNSQESVTEQDSKDSTYSLSSTLTLSKADYEKHKVYACEVTHQGLSSPVTKSFNRGEC

SEQ ID NO: 43 - protein, 103 aa, Artificial Sequence
  CD3 CH1
ASTKGPSVFPLAPSSKSTSGGTAALGCLVKDYFPEPVTVSWNSGALTSGVHTFPAVLQSSGLYSLSSVVTVPSSSLGTQTYICNVNHKPSNTKVDKKVEPKSC

SEQ ID NO: 44 - protein, 107 aa, Artificial Sequence
  CD3 CL
ASVAAPSVFIFPPSDEQLKSGTASVVCLLNNFYPREAKVQWKVDNALQSGNSQESVTEQDSKDSTYSLSSTLTLSKADYEKHKVYACEVTHQGLSSPVTKSFNRGEC

SEQ ID NO: 45 - protein, 671 aa, Artificial Sequence
  83A10 knob HC
EVQLLESGGGLVQPGGSLRLSCAASGFTFSSYAMSWVRQAPGKGLEWVSAISGSGGSTYYADSVKGRFTISRDNSKNTLYLQMNSLRAEDTAVYYCAKVLGWFDYWGQGTLVTVSSASTKGPSVFPLAPSSKSTSGGTAALGCLVEDYFPEPVTVSWNSGALTSGVHTFPAVLQSSGLYSLSSVVTVPSSSLGTQTYICNVNHKPSNTKVDEKVEPKSCDGGGGSGGGGSQAVVTQEPSLTVSPGGTVTLTCGSSTGAVTTSNYANWVQEKPGQAFRGLIGGTNKRAPGTPARFSGSLLGGKAALTLSGAQPEDEAEYYCALWYSNLWVFGGGTKLTVLSSASTKGPSVFPLAPSSKSTSGGTAALGCLVKDYFPEPVTVSWNSGALTSGVHTFPAVLQSSGLYSLSSVVTVPSSSLGTQTYICNVNHKPSNTKVDKKVEPKSCDKTHTCPPCPAPEAAGGPSVFLFPPKPKDTLMISRTPEVTCVVVDVSHEDPEVKFNWYVDGVEVHNAKTKPREEQYNSTYRVVSVLTVLHQDWLNGKEYKCKVSNKALGAPIEKTISKAKGQPREPQVYTLPPCRDELTKNQVSLWCLVKGFYPSDIAVEWESNGQPENNYKTTPPVLDSDGSFFLYSKLTVDKSRWQQGNVFSCSVMHEALHNHYTQKSLSLSPGK

SEQ ID NO: 46 - protein, 446 aa, Artificial Sequence
  83A10 hole HC
EVQLLESGGGLVQPGGSLRLSCAASGFTFSSYAMSWVRQAPGKGLEWVSAISGSGGSTYYADSVKGRFTISRDNSKNTLYLQMNSLRAEDTAVYYCAKVLGWFDYWGQGTLVTVSSASTKGPSVFPLAPSSKSTSGGTAALGCLVEDYFPEPVTVSWNSGALTSGVHTFPAVLQSSGLYSLSSVVTVPSSSLGTQTYICNVNHKPSNTKVDEKVEPKSCDKTHTCPPCPAPEAAGGPSVFLFPPKPKDTLMISRTPEVTCVVVDVSHEDPEVKFNWYVDGVEVHNAKTKPREEQYNSTYRVVSVLTVLHQDWLNGKEYKCKVSNKALGAPIEKTISKAKGQPREPQVCTLPPSRDELTKNQVSLSCAVKGFYPSDIAVEWESNGQPENNYKTTPPVLDSDGSFFLVSKLTVDKSRWQQGNVFSCSVMHEALHNHYTQKSLSLSPGK

SEQ ID NO: 47 - protein, 216 aa, Artificial Sequence
  83A10 LC
EIVLTQSPGTLSLSPGERATLSCRASQSVSSSYLAWYQQKPGQAPRLLIYGASSRATGIPDRFSGSGSGTDFTLTISRLEPEDFAVYYCQQYGYPPDFTFGQGTKVEIKRTVAAPSVFIFPPSDRKLKSGTASVVCLLNNFYPREAKVQWKVDNALQSGNSQESVTEQDSKDSTYSLSSTLTLSKADYEKHKVYACEVTHQGLSSPVTKSFNRGEC

SEQ ID NO: 48 - protein, 232 aa, Artificial Sequence
  CD3 LC
EVQLLESGGGLVQPGGSLRLSCAASGFTFSTYAMNWVRQAPGKGLEWVSRIRSKYNNYATYYADSVKGRFTISRDDSKNTLYLQMNSLRAEDTAVYYCVRHGNFGNSYVSWFAYWGQGTLVTVSSASVAAPSVFIFPPSDEQLKSGTASVVCLLNNFYPREAKVQWKVDNALQSGNSQESVTEQDSKDSTYSLSSTLTLSKADYEKHKVYACEVTHQGLSSPVTKSFNRGEC

SEQ ID NO: 49 - protein, 671 aa, Artificial Sequence
  Mab21 knob HC
EVQLLESGGGLVQPGGSLRLSCAASGFTFSDNAMGWVRQAPGKGLEWVSAISGPGSSTYYADSVKGRFTISRDNSKNTLYLQMNSLRAEDTAVYYCAKVLGWFDYWGQGTLVTVSSASTKGPSVFPLAPSSKSTSGGTAALGCLVEDYFPEPVTVSWNSGALTSGVHTFPAVLQSSGLYSLSSVVTVPSSSLGTQTYICNVNHKPSNTKVDEKVEPKSCDGGGGSGGGGSQAVVTQEPSLTVSPGGTVTLTCGSSTGAVTTSNYANWVQEKPGQAFRGLIGGTNKRAPGTPARFSGSLLGGKAALTLSGAQPEDEAEYYCALWYSNLWVFGGGTKLTVLSSASTKGPSVFPLAPSSKSTSGGTAALGCLVKDYFPEPVTVSWNSGALTSGVHTFPAVLQSSGLYSLSSVVTVPSSSLGTQTYICNVNHKPSNTKVDKKVEPKSCDKTHTCPPCPAPEAAGGPSVFLFPPKPKDTLMISRTPEVTCVVVDVSHEDPEVKFNWYVDGVEVHNAKTKPREEQYNSTYRVVSVLTVLHQDWLNGKEYKCKVSNKALGAPIEKTISKAKGQPREPQVYTLPPCRDELTKNQVSLWCLVKGFYPSDIAVEWESNGQPENNYKTTPPVLDSDGSFFLYSKLTVDKSRWQQGNVFSCSVMHEALHNHYTQKSLSLSPGK

SEQ ID NO: 50 - protein, 446 aa, Artificial Sequence
  Mab21 hole HC
EVQLLESGGGLVQPGGSLRLSCAASGFTFSDNAMGWVRQAPGKGLEWVSAISGPGSSTYYADSVKGRFTISRDNSKNTLYLQMNSLRAEDTAVYYCAKVLGWFDYWGQGTLVTVSSASTKGPSVFPLAPSSKSTSGGTAALGCLVEDYFPEPVTVSWNSGALTSGVHTFPAVLQSSGLYSLSSVVTVPSSSLGTQTYICNVNHKPSNTKVDEKVEPKSCDKTHTCPPCPAPEAAGGPSVFLFPPKPKDTLMISRTPEVTCVVVDVSHEDPEVKFNWYVDGVEVHNAKTKPREEQYNSTYRVVSVLTVLHQDWLNGKEYKCKVSNKALGAPIEKTISKAKGQPREPQVCTLPPSRDELTKNQVSLSCAVKGFYPSDIAVEWESNGQPENNYKTTPPVLDSDGSFFLVSKLTVDKSRWQQGNVFSCSVMHEALHNHYTQKSLSLSPGK

SEQ ID NO: 51 - protein, 216 aa, Artificial Sequence
  Mab21 LC
EIVLTQSPGTLSLSPGERATLSCRASQSVSEYYLAWYQQKPGQAPRLLIEHASTRATGIPDRFSGSGSGTDFTLTISRLEPEDFAVYYCQQYGYPPDFTFGQGTKVEIKRTVAAPSVFIFPPSDRKLKSGTASVVCLLNNFYPREAKVQWKVDNALQSGNSQESVTEQDSKDSTYSLSSTLTLSKADYEKHKVYACEVTHQGLSSPVTKSFNRGEC

SEQ ID NO: 52 - protein, 671 aa, Artificial Sequence; identical to SEQ ID NO: 49
  Mab22 knob HC

SEQ ID NO: 53 - protein, 446 aa, Artificial Sequence; identical to SEQ ID NO: 50
  Mab22 hole HC

SEQ ID NO: 54 - protein, 216 aa, Artificial Sequence
  Mab22 LC
EIVLTQSPGTLSLSPGERATLSCRASQSVSSYYLAWYQQKPGQAPRLLISGAGSRATGIPDRFSGSGSGTDFTLTISRLEPEDFAVYYCQQYGYPPDFTFGQGTKVEIKRTVAAPSVFIFPPSDRKLKSGTASVVCLLNNFYPREAKVQWKVDNALQSGNSQESVTEQDSKDSTYSLSSTLTLSKADYEKHKVYACEVTHQGLSSPVTKSFNRGEC

SEQ ID NO: 55 - protein, 671 aa, Artificial Sequence; identical to SEQ ID NO: 49
  Mab42 knob HC

SEQ ID NO: 56 - protein, 446 aa, Artificial Sequence; identical to SEQ ID NO: 50
  Mab42 hole HC

SEQ ID NO: 57 - protein, 216 aa, Artificial Sequence
  Mab42 LC
EIVLTQSPGTLSLSPGERATLSCRASQSVSDEYLSWYQQKPGQAPRLLIHSASTRATGIPDRFSGSGSGTDFTLAISRLEPEDFAVYYCQQYGYPPDFTFGQGTKVEIKRTVAAPSVFIFPPSDRKLKSGTASVVCLLNNFYPREAKVQWKVDNALQSGNSQESVTEQDSKDSTYSLSSTLTLSKADYEKHKVYACEVTHQGLSSPVTKSFNRGEC